European Patent Application EP 4 755 401 A1, published June 10, 2026. Title: 一种含有糖皮质激素的抗体药物偶联物的药物组合物. Applicant: 江苏恒瑞医药股份有限公司. The sequence listing filed with the application follows.

SEQUENCE LISTING (13 sequences)

SEQ ID NO: 1 - protein, 5 aa, synthetic construct
DYGMH

SEQ ID NO: 2 - protein, 17 aa, synthetic construct
FISSGSSIIYYADIVKG

SEQ ID NO: 3 - protein, 9 aa, synthetic construct
GNKRGFFDY

SEQ ID NO: 4 - protein, 10 aa, synthetic construct
RASSSVPYMY

SEQ ID NO: 5 - protein, 7 aa, synthetic construct
LTSNLAS

SEQ ID NO: 6 - protein, 11 aa, synthetic construct
QQWRAYPPMLT

SEQ ID NO: 7 - protein, 108 aa, synthetic construct
EIVLTQSPATLSLSPGERATLSCRASSSVPYMYWYQQKPGQAPRLLIYLTSNLASGIPARFSGSGSGTDFTLTISSLEPEDFAVYYCQQWRAYPPMLTFGGGTKVEIK

SEQ ID NO: 8 - protein, 118 aa, synthetic construct
EVQLVESGGGLVQPGGSLRLSCAASGFTFSDYGMHWVRQAPGKGLEWVAFISSGSSIIYYADIVKGRSTISRDNAKNTLYLQMNSLRAEDTAVYYCTRGNKRGFFDYWGQGTLVTVSS

SEQ ID NO: 9 - protein, 445 aa, synthetic construct
EVQLVESGGGLVQPGGSLRLSCAASGFTFSDYGMHWVRQAPGKGLEWVAFISSGSSIIYYADIVKGRSTISRDNAKNTLYLQMNSLRAEDTAVYYCTRGNKRGFFDYWGQGTLVTVSSASTKGPSVFPLAPCSRSTSESTAALGCLVKDYFPEPVTVSWNSGALTSGVHTFPAVLQSSGLYSLSSVVTVPSSSLGTKTYTCNVDHKPSNTKVDKRVESKYGPPCPPCPAPEFLGGPSVFLFPPKPKDTLMISRTPEVTCVVVDVSQEDPEVQFNWYVDGVEVHNAKTKPREEQFNSTYRVVSVLTVLHQDWLNGKEYKCKVSNKGLPSSIEKTISKAKGQPREPQVYTLPPSQEEMTKNQVSLTCLVKGFYPSDIAVEWESNGQPENNYKTTPPVLDSDGSFFLYSRLTVDKSRWQEGNVFSCSVMHEALHNHYTQKSLSLSLGK

SEQ ID NO: 10 - protein, 215 aa, synthetic construct
EIVLTQSPATLSLSPGERATLSCRASSSVPYMYWYQQKPGQAPRLLIYLTSNLASGIPARFSGSGSGTDFTLTISSLEPEDFAVYYCQQWRAYPPMLTFGGGTKVEIKRTVAAPSVFIFPPSDEQLKSGTASVVCLLNNFYPREAKVQWKVDNALQSGNSQESVTEQDSKDSTYSLSSTLTLSKADYEKHKVYACEVTHQGLSSPVTKSFNRGEC

SEQ ID NO: 11 - protein, 216 aa, synthetic construct
EVQLVESGGGLVQPGGSLRLSCAASGFTFSDYGMHWVRQAPGKGLEWVAFISSGSSIIYYADIVKGRSTISRDNAKNTLYLQMNSLRAEDTAVYYCTRGNKRGFFDYWGQGTLVTVSSASTKGPSVFPLAPCSRSTSESTAALGCLVKDYFPEPVTVSWNSGALTSGVHTFPAVLQSSGLYSLSSVVTVPSSSLGTKTYTCNVDHKPSNTKVDKRV

SEQ ID NO: 12 - protein, 10 aa, synthetic construct
GFTFSDYGMH

SEQ ID NO: 13 - protein, 160 aa, synthetic construct
ASDEEIQDVSGTWYLKAMTVDSRCPRAVYNSVTPMTLTTLEGGNLEAKFTAQRKGRWQKYKLVLEKTDEPGKYTASGGRHVAYIIRSHVKDHYIFHSEGLCPGQPVPGVWLVGRDPKNNLEALEDFEKAAGARGLSTESILIPRQSETSSPGSDHHHHHH